European Patent Specification EP 3 624 828 B1, published August 7, 2024. Title: PHARMACEUTICAL FORMULATION COMPRISING INCRETIN-INSULIN CONJUGATES. Applicant: Shi, Shuai Antochshuk, Valentyn. Application 62/507,964. The sequence listing filed with the application follows.

SEQUENCE LISTING (20 sequences)

SEQ ID NO: 1 - protein, 40 aa, Artificial Sequence
  Incretin portion of formula I
  MISC_FEATURE (1)..(1): X1 is His, Tyr, or absent
  MISC_FEATURE (2)..(2): X2 is aminoisobutyric acid
  MISC_FEATURE (3)..(3): X3 is Glu or Gln
  MISC_FEATURE (5)..(5): X5 is Thr or Ile
  MISC_FEATURE (10)..(10): X10 is Tyr or Lys acylated with a C16 to C20 alkyl group optionally via a gamma Glu linker
  MISC_FEATURE (12)..(12): X12 is Ile or Arg
  MISC_FEATURE (16)..(16): X16 is Lys, Arg, or Glu
  MISC_FEATURE (17)..(17): X17 is Gln or Arg
  MISC_FEATURE (20)..(20): X20 is Gln or aminoisobutyric acid
  MISC_FEATURE (21)..(21): X21 is Glu or Asp
  MISC_FEATURE (24)..(24): X24 is Asn, Gln, or Ala
  MISC_FEATURE (28)..(28): X28 is Ala or Asp
  MISC_FEATURE (29)..(29): X29 is Ala or Gly
  MISC_FEATURE (40)..(40): X40 is absent, or Lys, or Lys acylated with a C16 to C20 alkyl group optionally via a gamma Glu
XXXGXFTSDXSXYLDXXAAXXFVXWLLXXGPSSGAPPPSX

SEQ ID NO: 2 - protein, 21 aa, Homo sapiens
GIVEQCCTSICSLYQLENYCN

SEQ ID NO: 3 - protein, 30 aa, Homo sapiens
FVNQHLCGSHLVEALYLVCGERGFFYTPKT

SEQ ID NO: 4 - protein, 39 aa, Artificial Sequence
  Incretin peptide of Compound 99
  MISC_FEATURE (2)..(2): wherein X2 and X20 are each independently aminoisobutyric acid
  MISC_FEATURE (20)..(20): wherein X2 and X20 are each independently aminoisobutyric acid
YXEGTFTSDYSIYLDKQAAXEFVNWLLAGGPSSGAPPPS

SEQ ID NO: 5 - protein, 39 aa, Artificial Sequence
  Incretin peptide of Compound 100
  MISC_FEATURE (2)..(2): wherein X2 is aminoisobutyric acid
  MISC_FEATURE (10)..(10): wherein X10 is Lys acylated with a C16 fatty acyl group via gamma-Glu spacer
  MISC_FEATURE (20)..(20): wherein X20 is aminoisobutyric acid
YXEGTFTSDXSIYLDKQAAXEFVNWLLAGGPSSGAPPPS

SEQ ID NO: 6 - protein, 40 aa, Artificial Sequence
  Incretin peptide of Compound 101
  MISC_FEATURE (2)..(2): wherein X2 is aminoisobutyric acid
  MISC_FEATURE (20)..(20): wherein X20 is aminoisobutyric acid
  MISC_FEATURE (40)..(40): wherein X40 is Lys acylated with a C16 fatty acyl group via gamma-Glu spacer
YXEGTFTSDYSIYLDKQAAXEFVNWLLAGGPSSGAPPPSX

SEQ ID NO: 7 - protein, 39 aa, Artificial Sequence
  Incretin peptide of Compound 102
  MISC_FEATURE (2)..(2): wherein X2 is aminoisobutyric acid
  MISC_FEATURE (10)..(10): wherein X10 is Lys acylated with a C16 fatty acyl group via gamma-Glu spacer
HXEGTFTSDXSRYLDERAAQEFVAWLLDAGPSGAPPPSK

SEQ ID NO: 8 - protein, 39 aa, Artificial Sequence
  Incretin peptide of Compound 103
  MISC_FEATURE (2)..(2): wherein X2 is aminoisobutyric acid
  MISC_FEATURE (10)..(10): wherein X10 is Lys acylated with a C16 fatty acyl group via gamma-Glu spacer
HXQGTFTSDXSRYLDERAAQDFVQWLLDAGPSGAPPPSK

SEQ ID NO: 9 - protein, 39 aa, Artificial Sequence
  Incretin peptide of Compound 104
  MISC_FEATURE (2)..(2): wherein X2 is aminoisobutyric acid
  MISC_FEATURE (10)..(10): wherein X10 is Lys acylated with a C16 fatty acyl group via gamma-Glu spacer
HXQGTFTSDXSRYLDERAAQDFVQWLLDGGPSGAPPPSK

SEQ ID NO: 10 - protein, 39 aa, Artificial Sequence
  Incretin peptide of Compound 105
  MISC_FEATURE (2)..(2): wherein X2 is aminoisobutyric acid
  MISC_FEATURE (10)..(10): wherein X10 is Lys acylated with a C16 fatty acyl group via gamma-Glu spacer
HXEGTFTSDXSRYLDERAAQDFVQWLLDGGPSGAPPPSK

SEQ ID NO: 11 - protein, 37 aa, Artificial Sequence
  Incretin peptide of Compound 106
  MISC_FEATURE (1)..(1): wherein X1 is aminoisobutyric acid
  MISC_FEATURE (9)..(9): wherein X9 is Lys acylated with a C16 fatty acyl group via gamma-Glu spacer
  MISC_FEATURE (19)..(19): wherein X19 is aminoisobutyric acid
XEGTFTSDXSIYLDKQAAXEFVNWLLAGGPSGAPPPS

SEQ ID NO: 12 - protein, 40 aa, Artificial Sequence
  Incretin peptide of Compound 99 including Cysteine of linker
  MISC_FEATURE (2)..(2): wherein X2 is aminoisobutyric acid
  MISC_FEATURE (20)..(20): wherein X20 is aminoisobutyric acid
YXEGTFTSDYSIYLDKQAAXEFVNWLLAGGPSSGAPPPSC

SEQ ID NO: 13 - protein, 40 aa, Artificial Sequence
  Incretin peptide of Compound 100 including Cysteine of linker
  MISC_FEATURE (2)..(2): wherein X2 is aminoisobutyric acid
  MISC_FEATURE (10)..(10): wherein X10 is Lys acylated with a C16 fatty acyl group via gamma-Glu spacer
  MISC_FEATURE (20)..(20): wherein X20 is aminoisobutyric acid
YXEGTFTSDXSIYLDKQAAXEFVNWLLAGGPSSGAPPPSC

SEQ ID NO: 14 - protein, 41 aa, Artificial Sequence
  Incretin peptide of Compound 101 including Cysteine of linker
  MISC_FEATURE (2)..(2): wherein X2 is aminoisobutyric acid
  MISC_FEATURE (20)..(20): wherein X20 is aminoisobutyric acid
  MISC_FEATURE (40)..(40): wherein X40 is Lys acylated with a C16 fatty acyl group via gamma-Glu spacer
YXEGTFTSDYSIYLDKQAAXEFVNWLLAGGPSSGAPPPSXC

SEQ ID NO: 15 - protein, 40 aa, Artificial Sequence
  Incretin peptide of Compound 102 including Cysteine of linker
  MISC_FEATURE (2)..(2): wherein X2 is aminoisobutyric acid
  MISC_FEATURE (10)..(10): wherein X10 is Lys acylated with a C16 fatty acyl group via gamma-Glu spacer
HXEGTFTSDXSRYLDERAAQEFVAWLLDAGPSGAPPPSKC

SEQ ID NO: 16 - protein, 40 aa, Artificial Sequence
  Incretin peptide of Compound 103 including Cysteine of linker
  MISC_FEATURE (2)..(2): wherein X2 is aminoisobutyric acid
  MISC_FEATURE (10)..(10): wherein X10 is Lys acylated with a C16 fatty acyl group via gamma-Glu spacer
HXQGTFTSDXSRYLDERAAQDFVQWLLDAGPSGAPPPSKC

SEQ ID NO: 17 - protein, 40 aa, Artificial Sequence
  Incretin peptide of Compound 104 including Cysteine of linker
  MISC_FEATURE (2)..(2): wherein X2 is aminoisobutyric acid
  MISC_FEATURE (10)..(10): wherein X10 is Lys acylated with a C16 fatty acyl group via gamma-Glu spacer
HXQGTFTSDXSRYLDERAAQDFVQWLLDGGPSGAPPPSKC

SEQ ID NO: 18 - protein, 40 aa, Artificial Sequence
  Incretin peptide of Compound 105 including Cysteine of linker
  MISC_FEATURE (2)..(2): wherein X2 is aminoisobutyric acid
  MISC_FEATURE (10)..(10): wherein X10 is Lys acylated with a C16 fatty acyl group via gamma-Glu spacer
HXEGTFTSDXSRYLDERAAQDFVQWLLDGGPSGAPPPSKC

SEQ ID NO: 19 - protein, 38 aa, Artificial Sequence
  Incretin peptide of Compound 106 including Cysteine of linker
  MISC_FEATURE (1)..(1): wherein X1 is aminoisobutyric acid
  MISC_FEATURE (9)..(9): wherein X9 is Lys acylated with a C16 fatty acyl group via gamma-Glu spacer
  MISC_FEATURE (19)..(19): wherein X19 is aminoisobutyric acid
XEGTFTSDXSIYLDKQAAXEFVNWLLAGGPSGAPPPSC

SEQ ID NO: 20 - protein, 41 aa, Artificial Sequence
  Incretin peptide of formula I including Cysteine of linker
  MISC_FEATURE (1)..(1): X1 is His, Tyr, or absent
  MISC_FEATURE (2)..(2): X2 is aminoisobutyric acid
  MISC_FEATURE (3)..(3): X3 is Glu or Gln
  MISC_FEATURE (5)..(5): X5 is Thr or Ile
  MISC_FEATURE (10)..(10): X10 is Tyr or Lys acylated with a C16 to C20 alkyl group optionally via a gamma Glu linker
  MISC_FEATURE (12)..(12): X12 is Ile or Arg
  MISC_FEATURE (16)..(16): X16 is Lys, Arg, or Glu
  MISC_FEATURE (17)..(17): X17 is Gln or Arg
  MISC_FEATURE (20)..(20): X20 is Gln or aminoisobutyric acid
  MISC_FEATURE (21)..(21): X21 is Glu or Asp
  MISC_FEATURE (24)..(24): X24 is Asn, Gln, or Ala
  MISC_FEATURE (28)..(28): X28 is Ala or Asp
  MISC_FEATURE (29)..(29): X29 is Ala or Gly
  MISC_FEATURE (40)..(40): X40 is absent, or Lys, or Lys acylated with a C16 to C20 alkyl group optionally via a gamma Glu
XXXGXFTSDXSXYLDXXAAXXFVXWLLXXGPSSGAPPPSXC